European Patent Application EP 4 378 956 A1, published June 5, 2024. Title: B7H6抗体及其应用. Applicant: 合肥天港免疫药物有限公司. Application CN. The sequence listing filed with the application follows.

SEQUENCE LISTING (66 sequences)

SEQ ID NO: 1 - protein, 8 aa, synthetic construct
GYTFTSYY

SEQ ID NO: 2 - protein, 8 aa, synthetic construct
INPSNGGT

SEQ ID NO: 3 - protein, 14 aa, synthetic construct
TRTLYYGNDWYFDV

SEQ ID NO: 4 - protein, 5 aa, synthetic construct
SSVNY

SEQ ID NO: 5 - skipped

SEQ ID NO: 6 - protein, 9 aa, synthetic construct
QQWSSNPVT

SEQ ID NO: 7 - protein, 8 aa, synthetic construct
GYTFTDYN

SEQ ID NO: 8 - protein, 8 aa, synthetic construct
INPNNGGT

SEQ ID NO: 9 - protein, 13 aa, synthetic construct
ARSEVFYGNYADY

SEQ ID NO: 10 - protein, 10 aa, synthetic construct
QSVDYDGDSY

SEQ ID NO: 11 - skipped

SEQ ID NO: 12 - protein, 9 aa, synthetic construct
QQSKEDPRT

SEQ ID NO: 13 - protein, 121 aa, synthetic construct
QVQLQQSGAELVKPGASVKLSCKASGYTFTSYYMYWVKQRPGQGLEWIGEINPSNGGTNFNEKFKSKATLTVDKSSSTAYMQLSSLTSEDSAVYYCTRTLYYGNDWYFDVWGAGTTVTVSS

SEQ ID NO: 14 - protein, 106 aa, synthetic construct
QIVLTQSPAIMSASPGEKVTMTCSASSSVNYMHWYQQKSGTSPKRWIYDTSKLASGVPARFSGSGSGTSYSLTISSMEAEDAATYYCQQWSSNPVTFGAGTKLELK

SEQ ID NO: 15 - protein, 120 aa, synthetic construct
EVLLQQSGPEVVKPGASVKITCKASGYTFTDYNMDWVKQSHGKSLEWIGDINPNNGGTLYNQKFRGRVTLIVDKSSSTAYMELRSLTSDDTAVYYCARSEVFYGNYADYWGQGTTLTVSS

SEQ ID NO: 16 - protein, 111 aa, synthetic construct
DIVLTQSPVSLAVPLGQRATISCKASQSVDYDGDSYMNWYQQKPGQPPKLLIYAASTLHSGIPVRFSGSGSGTDFTLNIHPVEEEDAASYYCQQSKEDPRTFGGGTKLEIK

SEQ ID NO: 17 - protein, 121 aa, synthetic construct
EVQLVQSGAEVKKPGASVKVSCKASGYTFTSYYMYWVRQAPGQGLEWIGEINPSNGGTNFNEKFKSRVTLTVDKSISTAYMELSRLRSDDTAVYYCTRTLYYGNDWYFDVWGQGTTVTVSS

SEQ ID NO: 18 - protein, 106 aa, synthetic construct
EIVLTQSPDFQSVTPKEKVTITCSASSSVNYMHWYQQKPDQSPKRLIYDTSKLASGVPSRFSGSGSGTDYTLTINSLEAEDAATYYCQQWSSNPVTFGQGTKLEIK

SEQ ID NO: 19 - protein, 120 aa, synthetic construct
EVQLVQSGAEVKKPGASVKVSCKASGYTFTDYNMDWVRQAPGKGLEWIGDINPNNGGTLYNQKFRGRVTLTVDKSISTAYMELSRLRSDDTAVYYCARSEVFYGNYADYWGQGTTVTVSS

SEQ ID NO: 20 - protein, 111 aa, synthetic construct
DIVLTQTPLSLSVTPGQPASISCKASQSVDYDGDSYMNWYLQKPGQPPQLLIYAASTLHSGVPDRFSGSGSGTDFTLKISRVEAEDVGVYYCQQSKEDPRTFGQGTKLEIK

SEQ ID NO: 21 - protein, 454 aa, synthetic construct
MTWRAAASTCAALLILLWALTTEGDLKVEMMAGGTQITPLNDNVTIFCNIFYSQPLNITSMGITWFWKSLTFDKEVKVFEFFGDHQEAFRPGAIVSPWRLKSGDASLRLPGIQLEEAGEYRCEVVVTPLKAQGTVQLEVVASPASRLLLDQVGMKENEDKYMCESSGFYPEAINITWEKQTQKFPHPIEISEDVITGPTIKNMDGTFNVTSCLKLNSSQEDPGTVYQCVVRHASLHTPLRSNFTLTAARHSLSETEKTDNFSIHWWPISFIGVGLVLLIVLIPWKKICNKSSSAYTPLKCILKHWNSFDTQTLKKEHLIFFCTRAWPSYQLQDGEAWPPEGSVNINTIQQLDVFCRQEGKWSEVPYVQAFFALRDNPDLCQCCRIDPALLTVTSGKSIDDNSTKSEKQTPREHSDAVPDAPILPVSPIWEPPPATTSTTPVLSSQPPTLLLPLQ

SEQ ID NO: 22 - protein, 471 aa, synthetic construct
DLKVEMMAGGTQITPLNDNVTIFCNIFYSQPLNITSMGITWFWKSLTFDKEVKVFEFFGDHQEAFRPGAIVSPWRLKSGDASLRLPGIQLEEAGEYRCEVVVTPLKAQGTVQLEVVASPASRLLLDQVGMKENEDKYMCESSGFYPEAINITWEKQTQKFPHPIEISEDVITGPTIKNMDGTFNVTSCLKLNSSQEDPGTVYQCVVRHASLHTPLRSNFTLTAARHSLSETEKTDNFSLEPKSCDKTHTCPPCPAPELLGGPSVFLFPPKPKDTLMISRTPEVTCVVVDVSHEDPEVKFNWYVDGVEVHNAKTKPREEQYNSTYRVVSVLTVLHQDWLNGKEYKCKVSNKALPAPIEKTISKAKGQPREPQVYTLPPSREEMTKNQVSLTCLVKGFYPSDIAVEWESNGQPENNYKTTPPVLDSDGSFFLYSKLTVDKSRWQQGNVFSCSVMHEALHNHYTQKSLSLSPGK

SEQ ID NO: 23 - protein, 466 aa, synthetic construct
DLKVEMMARGIQATRLNDSVTISCKVIYSQPLNITSMGITWFRKSLTLDKEVKVFEFFGDHQKAFRPGANVSLWRLKSGDASLKLPGVQLEEAGEYRCEVVVTPLKAQGTVQLKVVASPTSRLFQDQAVVKENEGKYMCESSRFYPKDINITWEKWTQKSPHHVVISENVITGPTIKNMDGTFNITSYLKLNSSQEDPGTVYRCVIRHESLHTPVSIDFILTAPQQSLSEPEKTDPKSCDKTHTCPPCPAPELLGGPSVFLFPPKPKDTLMISRTPEVTCVVVDVSHEDPEVKFNWYVDGVEVHNAKTKPREEQYNSTYRVVSVLTVLHQDWLNGKEYKCKVSNKALPAPIEKTISKAKGQPREPQVYTLPPSRDELTKNQVSLTCLVKGFYPSDIAVEWESNGQPENNYKTTPPVLDSDGSFFLYSKLTVDKSRWQQGNVFSCSVMHEALHNHYTQKSLSLSPGK

SEQ ID NO: 24 - protein, 296 aa, synthetic construct
MAWRAASSACAAPLLLWCALMTAGDLKVEMMARGIQATRLNDSVTISCKVIYSQPLNITSMGITWFRKSLTLDKEVKVFEFFGDHQKAFRPGANVSLWRLKSGDASLKLPGVQLEEAGEYRCEVVVTPLKAQGTVQLKVVASPTSRLFQDQAVVKENEGKYMCESSRFYPKDINITWEKWTQKSPHHVVISENVITGPTIKNMDGTFNITSYLKLNSSQEDPGTVYRCVIRHESLHTPVSIDFILTAPQQSLSEPEKTDIFSIYGWLFSFIAAGLILLIVLIHWKKVPLREEEGRN

SEQ ID NO: 25 - protein, 356 aa, synthetic construct
WVSQPPEIRTLEGSSAFLPCSFNASQGRLAIGSVTWFRDEVVPGKEVRNGTPEFRGRLAPLASSRFLHDHQAELHIRDVRGHDASIYVCRVEVLGLGVGTGNGTRLVVEKEHPQLGENLYFQSLEPKSCDKTHTCPPCPAPELLGGPSVFLFPPKPKDTLMISRTPEVTCVVVDVSHEDPEVKFNWYVDGVEVHNAKTKPREEQYNSTYRVVSVLTVLHQDWLNGKEYKCKVSNKALPAPIEKTISKAKGQPREPQVYTLPPSREEMTKNQVSLTCLVKGFYPSDIAVEWESNGQPENNYKTTPPVLDSDGSFFLYSKLTVDKSRWQQGNVFSCSVMHEALHNHYTQKSLSLSPGK

SEQ ID NO: 26 - protein, 451 aa, synthetic construct
QVQLQQSGAELVKPGASVKLSCKASGYTFTSYYMYWVKQRPGQGLEWIGEINPSNGGTNFNEKFKSKATLTVDKSSSTAYMQLSSLTSEDSAVYYCTRTLYYGNDWYFDVWGAGTTVTVSSAKTTAPSVYPLAPVCGDTTGSSVTLGCLVKGYFPEPVTLTWNSGSLSSGVHTFPAVLQSDLYTLSSSVTVTSSTWPSQSITCNVAHPASSTKVDKKIEPRGPTIKPCPPCKCPAPNLLGGPSVFIFPPKIKDVLMISLSPIVTCVVVDVSEDDPDVQISWFVNNVEVHTAQTQTHREDYNSTLRVVSALPIQHQDWMSGKEFKCKVNNKDLPAPIERTISKPKGSVRAPQVYVLPPPEEEMTKKQVTLTCMVTDFMPEDIYVEWTNNGKTELNYKNTEPVLDSDGSYFMYSKLRVEKKNWVERNSYSCSVVHEGLHNHHTTKSFSRTPGK

SEQ ID NO: 27 - protein, 213 aa, synthetic construct
QIVLTQSPAIMSASPGEKVTMTCSASSSVNYMHWYQQKSGTSPKRWIYDTSKLASGVPARFSGSGSGTSYSLTISSMEAEDAATYYCQQWSSNPVTFGAGTKLELKRADAAPTVSIFPPSSEQLTSGGASVVCFLNNFYPKDINVKWKIDGSERQNGVLNSWTDQDSKDSTYSMSSTLTLTKDEYERHNSYTCEATHKTSTSPIVKSFNRNEC

SEQ ID NO: 28 - protein, 450 aa, synthetic construct
EVLLQQSGPEVVKPGASVKITCKASGYTFTDYNMDWVKQSHGKSLEWIGDINPNNGGTLYNQKFRGRVTLIVDKSSSTAYMELRSLTSDDTAVYYCARSEVFYGNYADYWGQGTTLTVSSAKTTAPSVYPLAPVCGDTTGSSVTLGCLVKGYFPEPVTLTWNSGSLSSGVHTFPAVLQSDLYTLSSSVTVTSSTWPSQSITCNVAHPASSTKVDKKIEPRGPTIKPCPPCKCPAPNLLGGPSVFIFPPKIKDVLMISLSPIVTCVVVDVSEDDPDVQISWFVNNVEVHTAQTQTHREDYNSTLRVVSALPIQHQDWMSGKEFKCKVNNKDLPAPIERTISKPKGSVRAPQVYVLPPPEEEMTKKQVTLTCMVTDFMPEDIYVEWTNNGKTELNYKNTEPVLDSDGSYFMYSKLRVEKKNWVERNSYSCSVVHEGLHNHHTTKSFSRTPGK

SEQ ID NO: 29 - protein, 218 aa, synthetic construct
DIVLTQSPVSLAVPLGQRATISCKASQSVDYDGDSYMNWYQQKPGQPPKLLIYAASTLHSGIPVRFSGSGSGTDFTLNIHPVEEEDAASYYCQQSKEDPRTFGGGTKLEIKRADAAPTVSIFPPSSEQLTSGGASVVCFLNNFYPKDINVKWKIDGSERQNGVLNSWTDQDSKDSTYSMSSTLTLTKDEYERHNSYTCEATHKTSTSPIVKSFNRNEC

SEQ ID NO: 30 - protein, 451 aa, synthetic construct
EVQLVQSGAEVKKPGASVKVSCKASGYTFTSYYMYWVRQAPGQGLEWIGEINPSNGGTNFNEKFKSRVTLTVDKSISTAYMELSRLRSDDTAVYYCTRTLYYGNDWYFDVWGQGTTVTVSSASTKGPSVFPLAPSSKSTSGGTAALGCLVKDYFPEPVTVSWNSGALTSGVHTFPAVLQSSGLYSLSSVVTVPSSSLGTQTYICNVNHKPSNTKVDKKVEPKSCDKTHTCPPCPAPELLGGPSVFLFPPKPKDTLMISRTPEVTCVVVDVSHEDPEVKFNWYVDGVEVHNAKTKPREEQYNSTYRVVSVLTVLHQDWLNGKEYKCKVSNKALPAPIEKTISKAKGQPREPQVYTLPPSREEMTKNQVSLTCLVKGFYPSDIAVEWESNGQPENNYKTTPPVLDSDGSFFLYSKLTVDKSRWQQGNVFSCSVMHEALHNHYTQKSLSLSPGK

SEQ ID NO: 31 - protein, 213 aa, synthetic construct
EIVLTQSPDFQSVTPKEKVTITCSASSSVNYMHWYQQKPDQSPKRLIYDTSKLASGVPSRFSGSGSGTDYTLTINSLEAEDAATYYCQQWSSNPVTFGQGTKLEIKRTVAAPSVFIFPPSDEQLKSGTASVVCLLNNFYPREAKVQWKVDNALQSGNSQESVTEQDSKDSTYSLSSTLTLSKADYEKHKVYACEVTHQGLSSPVTKSFNRGEC

SEQ ID NO: 32 - protein, 450 aa, synthetic construct
EVQLVQSGAEVKKPGASVKVSCKASGYTFTDYNMDWVRQAPGKGLEWIGDINPNNGGTLYNQKFRGRVTLTVDKSISTAYMELSRLRSDDTAVYYCARSEVFYGNYADYWGQGTTVTVSSASTKGPSVFPLAPSSKSTSGGTAALGCLVKDYFPEPVTVSWNSGALTSGVHTFPAVLQSSGLYSLSSVVTVPSSSLGTQTYICNVNHKPSNTKVDKKVEPKSCDKTHTCPPCPAPELLGGPSVFLFPPKPKDTLMISRTPEVTCVVVDVSHEDPEVKFNWYVDGVEVHNAKTKPREEQYNSTYRVVSVLTVLHQDWLNGKEYKCKVSNKALPAPIEKTISKAKGQPREPQVYTLPPSREEMTKNQVSLTCLVKGFYPSDIAVEWESNGQPENNYKTTPPVLDSDGSFFLYSKLTVDKSRWQQGNVFSCSVMHEALHNHYTQKSLSLSPGK

SEQ ID NO: 33 - protein, 218 aa, synthetic construct
DIVLTQTPLSLSVTPGQPASISCKASQSVDYDGDSYMNWYLQKPGQPPQLLIYAASTLHSGVPDRFSGSGSGTDFTLKISRVEAEDVGVYYCQQSKEDPRTFGQGTKLEIKRTVAAPSVFIFPPSDEQLKSGTASVVCLLNNFYPREAKVQWKVDNALQSGNSQESVTEQDSKDSTYSLSSTLTLSKADYEKHKVYACEVTHQGLSSPVTKSFNRGEC

SEQ ID NO: 34 - DNA, 24 bp, synthetic construct
  source 1..24: mol_type = other DNA
gggtacacatttaccagctactat

SEQ ID NO: 35 - DNA, 24 bp, synthetic construct
  source 1..24: mol_type = other DNA
attaatccatctaacgggggaacc

SEQ ID NO: 36 - DNA, 42 bp, synthetic construct
  source 1..42: mol_type = other DNA
actaggaccctgtattacggtaacgactggtatttcgatgtg

SEQ ID NO: 37 - DNA, 15 bp, synthetic construct
  source 1..15: mol_type = other DNA
tcttctgttaactat

SEQ ID NO: 38 - skipped

SEQ ID NO: 39 - DNA, 27 bp, synthetic construct
  source 1..27: mol_type = other DNA
cagcaatggagcagtaatccagtcaca

SEQ ID NO: 40 - DNA, 24 bp, synthetic construct
  source 1..24: mol_type = other DNA
gggtacacatttacagactacaat

SEQ ID NO: 41 - DNA, 24 bp, synthetic construct
  source 1..24: mol_type = other DNA
atcaatccaaacaatggcggtacc

SEQ ID NO: 42 - DNA, 39 bp, synthetic construct
  source 1..39: mol_type = other DNA
gctcgctctgaagtcttttatgggaattatgctgactac

SEQ ID NO: 43 - DNA, 30 bp, synthetic construct
  source 1..30: mol_type = other DNA
cagagcgtggactatgatggcgacagctat

SEQ ID NO: 44 - skipped

SEQ ID NO: 45 - DNA, 27 bp, synthetic construct
  source 1..27: mol_type = other DNA
cagcagagcaaagaggatcctagaacc

SEQ ID NO: 46 - DNA, 363 bp, synthetic construct
  source 1..363: mol_type = other DNA
caggtgcagttgcaacaatctggtgcagagctggtgaaacctggtgcatcagtgaagctttcatgtaaagcttccgggtacacatttaccagctactatatgtactgggttaagcagcgtcctggacagggtctggagtggatcggcgagattaatccatctaacgggggaaccaactttaacgaaaagttcaagtctaaggctacactgacagtcgataaatcctcatccaccgcctacatgcagctctcttctctgacttcagaggacagcgccgtgtactactgcactaggaccctgtattacggtaacgactggtatttcgatgtgtggggtgccggtacaacagtgaccgtgtcctca

SEQ ID NO: 47 - DNA, 318 bp, synthetic construct
  source 1..318: mol_type = other DNA
caaatcgtgctgacccagtctccagcaataatgtccgcatctcctggtgagaaagtgaccatgacttgttcagcttcctcttctgttaactatatgcactggtaccaacagaagtctggcacctccccaaagcggtggatttatgacacctccaagctggctagcggggtacccgcaaggttctccggttcaggcagcggcacttcttactccctgactattagctctatggaggcagaggatgccgctacctactattgccagcaatggagcagtaatccagtcacatttggggccggaaccaagctggagctgaag

SEQ ID NO: 48 - DNA, 360 bp, synthetic construct
  source 1..360: mol_type = other DNA
gaagttctgcttcagcagtctggcccagaagttgttaagccaggagcctccgtgaaaattacttgcaaggcctccgggtacacatttacagactacaatatggactgggtgaagcagtcccatggaaagagtctggaatggatcggcgatatcaatccaaacaatggcggtaccctctataaccagaaatttcgcggacgtgtgaccttgatcgtcgacaaaagtagttctactgcctacatggagctgcgcagcctgactagtgacgacaccgccgtctactattgcgctcgctctgaagtcttttatgggaattatgctgactactggggccagggtaccactttgaccgtctccagt

SEQ ID NO: 49 - DNA, 333 bp, synthetic construct
  source 1..333: mol_type = other DNA
gacattgtgctgactcagagtcctgtaagtctggcagttcccctcggccaaagagctaccattagttgtaaggcttcccagagcgtggactatgatggcgacagctatatgaattggtatcaacagaagccaggacagccacccaagctgctgatctacgccgcctccaccctgcattcaggtatccctgtgcgattttctggtagtggctccggcacagatttcaccctgaatatccatccagttgaggaggaggatgctgcctcttactactgtcagcagagcaaagaggatcctagaaccttcggcggtggcactaagctggaaattaag

SEQ ID NO: 50 - DNA, 363 bp, synthetic construct
  source 1..363: mol_type = other DNA
gaagttcaactggttcagagcggagctgaggtaaagaagccaggtgccagcgtgaaagttagttgcaaggcatccggatacactttcactagctattatatgtattgggtgcgacaggccccagggcaaggtttggagtggatcggagagatcaatccttcaaatggcggcacaaatttcaacgaaaagttcaaatctcgcgtgactctgacagtggacaagtccatctccacagcatatatggagctgagccggcttagatccgatgacactgctgtctactattgtacaagaacactgtactatggcaacgactggtacttcgatgtctggggacaggggaccactgtgaccgtctccagt

SEQ ID NO: 51 - DNA, 318 bp, synthetic construct
  source 1..318: mol_type = other DNA
gaaatcgtgctgacccagagcccagatttccagagtgtcacaccaaaggagaaggtaacaattacatgcagtgccagcagtagcgtgaactatatgcattggtatcagcagaaacccgatcagtcccctaagcgactgatctacgatacctccaagctggccagcggtgttccaagtaggttctctggcagcgggtctgggacagactacactctcactatcaactctctggaagctgaggatgctgctacttattattgccagcagtggagctcaaatcccgttacctttggccagggtaccaagctcgaaattaaa

SEQ ID NO: 52 - DNA, 360 bp, synthetic construct
  source 1..360: mol_type = other DNA
gaagtgcagcttgtacagagtggagcagaggtcaagaaaccaggagcttccgtgaaggtgagctgcaaggcctccggctatacctttactgattacaacatggactgggtccgtcaggctcctggaaaaggactggagtggattggtgacattaatcctaataacggcggcacactttacaatcagaagtttcgtggtagagttacactgactgtggataaatcaatcagcaccgcctatatggagctgtcccgactgcggtccgacgatactgcagtgtattactgcgccaggtcagaggtgttttacggtaactacgcagactattggggccaggggacaacagtgacagtcagcagc

SEQ ID NO: 53 - DNA, 333 bp, synthetic construct
  source 1..333: mol_type = other DNA
gacatagtattgacccagacaccattgtctttgagcgttaccccaggccagccagcttcaatatcttgcaaggcctctcagtccgtcgactatgatggcgattcctacatgaattggtacctccaaaagccaggccaaccaccacagctgttgatttatgccgcttctacactccacagtggcgtgcccgatcgattttcaggatccggctcagggaccgatttcacccttaagatttctcgagtggaagccgaggatgtgggcgtgtattactgccagcagagcaaagaggatcctagaacttttggccagggaaccaagctggagattaaa

SEQ ID NO: 54 - DNA, 1365 bp, synthetic construct
  source 1..1365: mol_type = other DNA
atgacgtggagggctgccgcctccacgtgcgcggcgctcctgattctgctgtgggcgctgacgaccgaaggtgatctgaaagtagagatgatggcaggggggactcagatcacacccctgaatgacaatgtcaccatattctgcaatatcttttattcccaacccctcaacatcacgtctatgggtatcacctggttttggaagagtctgacgtttgacaaagaagtcaaagtctttgaattttttggagatcaccaagaggcattccgacctggagccattgtgtctccatggaggctgaagagtggggacgcctcactgcggctgcctggaatccagctggaggaagcaggagagtaccgatgtgaggtggtggtcacccctctgaaggcacagggaacagtccagcttgaagttgtggcttccccagccagcagattgttgctggatcaagtgggcatgaaagagaatgaagacaaatatatgtgtgagtcaagtgggttctacccagaggctattaatataacatgggagaagcagacccagaagtttccccatcccatagagatttctgaggatgtcatcactggtcccaccatcaagaatatggatggcacatttaatgtcactagctgcttgaagctgaactcctctcaggaagaccctgggactgtctaccagtgtgtggtacggcatgcgtccttgcatacccccttgaggagcaactttaccctgactgctgctcggcacagtctttctgaaactgagaagacagataatttttccattcattggtggcctatttcattcattggtgttggactggttttattaattgttttgattccttggaaaaagatatgtaacaaatcatcttcagcctatactcctctcaagtgcattctgaaacactggaactcctttgacactcagactctgaagaaagagcacctcatattcttttgcactcgggcatggccgtcttaccagctgcaggatggggaggcttggcctcctgagggaagtgttaatattaatactattcaacaactagatgttttctgcagacaggagggcaaatggtccgaggttccttatgtgcaagccttctttgccttgcgagacaacccagatctttgtcagtgttgtagaattgaccctgctctcctaacagttacatcaggcaagtccatagatgataattccacaaagtctgagaaacaaacccctagggaacactcggatgcagttccggatgccccaatccttcctgtctcccctatctgggaacctcctccagccacaacatcaacaactccagttctatcctcccaacccccaactttactgttacccctacagtaa

SEQ ID NO: 55 - DNA, 1413 bp, synthetic construct
  source 1..1413: mol_type = other DNA
gacctgaaggtggaaatgatggcagggggtactcagataacacctctcaatgataatgtcacaattttttgtaacatcttttactctcagccacttaatatcacctccatgggaatcacttggttttggaagtcattgaccttcgataaggaggtgaaggtatttgagtttttcggggaccaccaggaagctttccgaccaggagcaattgtgtccccttggcgcttgaagtctggcgacgccagcttgagacttcctggaatccaattggaggaagctggggagtacagatgtgaggttgtcgtgactcctctgaaagctcagggtaccgtgcagttggaggttgtcgcctcacccgcttcccggcttctgctggaccaggttggaatgaaggagaacgaagataagtatatgtgcgagagttccggattttatcccgaggccatcaacattacatgggagaaacagacccaaaagtttcctcaccccattgaaatcagcgaggatgtgattaccggacccaccattaaaaatatggatggcactttcaacgttacctcatgtttgaaattgaacagtagtcaggaagaccctggaacagtctatcagtgcgtcgtgagacacgcatccctccatacacctctgcgttcaaacttcactctcactgccgccaggcatagcctgagcgagaccgagaagaccgataacttctctctggagcctaagagctgcgacaagacccacacctgtccaccctgtccagcccctgagctgctgggggggccctccgtgttccttttccctccaaaacccaaggacaccctgatgatctctagaacccccgaagtcacatgcgtggtggtagatgtctctcatgaggaccccgaggtgaagttcaattggtacgtcgatggagtggaggtgcataacgccaagactaagcctagggaagagcagtataattcaacctaccgcgtcgtgtctgtgctcaccgtgctgcatcaagactggctcaacggcaaagaatacaagtgcaaggtctctaacaaggctctgcccgctcccatcgaaaagaccatctccaaggctaagggccaacccagggagccccaagtctacacactgcctccatcacgtgaagagatgactaaaaatcaagttagtttgacctgcttggttaagggcttctatccatctgatatagcagtcgaatgggagagcaacggccagcctgaaaacaactacaagacaactccacccgtcttggactccgacggtagttttttcctgtactccaaactgaccgtggataagagcagatggcagcagggcaacgtgttctcatgttccgtcatgcatgaagctctccacaaccactacacccagaagtctctgagtctctctcccggtaaa

SEQ ID NO: 56 - DNA, 1398 bp, synthetic construct
  source 1..1398: mol_type = other DNA
gatttgaaggtggagatgatggctcgaggaattcaggccaccagactcaacgacagcgtcacaatctcttgcaaagtgatctatagtcagcccctcaacataaccagtatgggaattacctggtttcgcaaatcactgactttggataaagaggttaaagtctttgaattttttggcgatcaccagaaggccttcagacccggagcaaatgtgtccctgtggaggctgaagtctggcgacgctagcctgaaacttccaggagttcagctcgaagaggccggcgagtacaggtgcgaagttgtagtaacccctctcaaagcacagggcaccgttcagctgaaggtggtggcttcacctacttctagacttttccaggatcaggccgtggttaaggagaacgagggcaaatatatgtgcgagtcctctcgtttttatcccaaagacatcaatatcacctgggagaaatggacacagaaatcacctcaccacgttgtaattagcgagaacgtgatcacaggccccacaataaagaacatggacggaactttcaatataacctcctacttgaagctgaactcctctcaagaagatcctggcactgtgtatagatgtgtgattaggcacgagagcctccacacacccgtctctattgacttcatattgactgcaccacagcagtctctgtctgaaccagaaaagaccgatccaaaatcctgtgacaagactcatacatgtcctccttgtccagcaccagagctgcttggtggccctagcgtgttcctgttccctcccaagcctaaggacaccctgatgatttcaagaacccccgaggtgacttgtgtggtcgtggatgtgagccacgaggatcctgaagtcaaattcaattggtacgttgatggcgtggaggtgcacaatgccaaaaccaagccacgagaggagcagtacaacagcacctacagagtggtgtctgtgctgaccgtgttgcatcaggactggcttaatggaaaagaatacaagtgtaaggtctccaataaagctctccctgccccaatcgagaagactatctctaaggctaaaggacagccaagggaaccccaggtttacacactgcccccaagccgagatgaattgacaaaaaatcaggtttccttgacctgcctggtgaagggtttctacccatctgatatcgccgttgagtgggagagcaatggacagcctgagaacaattacaaaacaacccctcctgtgttggatagtgatggcagcttctttctgtattctaagcttaccgtggataagtctagatggcagcaaggaaatgtgttttcctgcagcgtaatgcacgaagcacttcataatcattatacacagaagtctctctctcttagcccagggaag

SEQ ID NO: 57 - DNA, 888 bp, synthetic construct
  source 1..888: mol_type = other DNA
atggcatggagagctgcatcttccgcttgtgctgctcctttgcttctgtggtgtgctttgatgactgccggagacctgaaagtcgaaatgatggctagaggaatccaagctactcgcctgaatgatagtgtgacaatctcatgtaaagtaatttattcccagcctttgaacatcacctctatgggcattacctggtttcgcaagagtctcaccctggataaagaggtaaaagtgttcgagttctttggagaccatcaaaaagctttccgccctggagctaatgtgagcctttggcgcctgaagagtggagacgccagtctgaaattgcctggtgtgcagctcgaagaggctggtgaatataggtgcgaagtggtggtgactcctctgaaggctcaggggaccgtccagcttaaagtggtggccagtcctaccagtcgcctgtttcaggaccaggcagtggtcaaggagaacgaaggtaaatatatgtgtgaatcttctcgtttctacccaaaggatattaatatcacctgggagaagtggacccaaaagagcccacaccatgtggtcatctcagagaatgtgatcaccggccccaccatcaagaatatggatggaactttcaatatcacatcttacctgaagctgaattcaagccaagaggatcctggaaccgtatataggtgcgtcatcagacatgagagcctccacacacccgtgagcatcgacttcattctgacagctccacagcagagtctcagtgaacctgagaaaacagacattttttctatctatgggtggcttttttcttttatcgccgctgggctgatcttgctgatcgtgctcatccactggaaaaaagtgccactgcgagaagaagaaggcagaaac

SEQ ID NO: 58 - DNA, 1068 bp, synthetic construct
  source 1..1068: mol_type = other DNA
tgggtgagtcaaccacctgagattagaactctggagggcagctctgcattcttgccatgctccttcaacgcaagtcaggggaggctggctatcggttccgtaacatggtttagggatgaggtggtgccaggaaaagaagtgaggaacggaaccccagagttcagaggaagactggcccctctggcaagttcccgctttctgcatgatcaccaagccgaacttcacattcgcgacgtcagggggcacgacgcatctatatacgtgtgcagagtggaggtgcttggtctgggtgtgggcaccggaaacggcactcgactcgtcgttgagaaagagcatccacagctgggagaaaatctgtactttcagagcctcgaacctaagtcttgtgacaagacccatacctgtcctccctgtcctgctcctgaactgttggggggcccctctgtgttcctgttccctccaaagcccaaggacacactgatgattagcaggacaccagaagtcacatgtgtcgtggttgatgtgtcccacgaggatcccgaggttaaatttaattggtatgtggacggtgttgaggtgcataacgccaagaccaagcctcgagaagagcagtacaattccacttatagggtagtctccgtattgaccgtgctccatcaggactggctgaatggcaaagagtacaaatgcaaggtctccaataaggcccttccagccccaattgaaaagactatttcaaaggccaaggggcaacccagagagcctcaggtgtatacacttcctccctcacgtgaggagatgacaaagaaccaagtgagtctgacatgtctcgtgaaaggcttttacccttcagacattgctgtggagtgggaaagcaacggccaacccgagaacaactacaagaccacacctcccgtgctggacagcgatgggtctttctttctctacagcaagctgactgtggacaaaagtcgctggcagcaaggcaatgtcttcagctgctctgtgatgcacgaagccctccataatcattatacccagaagtctctgagcctgagcccaggaaag

SEQ ID NO: 59 - DNA, 1353 bp, synthetic construct
  source 1..1353: mol_type = other DNA
caggtgcagttgcaacaatctggtgcagagctggtgaaacctggtgcatcagtgaagctttcatgtaaagcttccgggtacacatttaccagctactatatgtactgggttaagcagcgtcctggacagggtctggagtggatcggcgagattaatccatctaacgggggaaccaactttaacgaaaagttcaagtctaaggctacactgacagtcgataaatcctcatccaccgcctacatgcagctctcttctctgacttcagaggacagcgccgtgtactactgcactaggaccctgtattacggtaacgactggtatttcgatgtgtggggtgccggtacaacagtgaccgtgtcctcagccaaaacaacagcccctagtgtatatccacttgcccctgtctgcggcgacactacagggtcttctgtgacactcgggtgtctggtcaaggggtatttccctgagccagtgaccctcacttggaactcaggctccctttctagcggcgtccacacatttccagccgtgcttcagtctgatctgtataccctgagcagcagcgtgaccgtcacctcctccacatggccttcacaaagcataacttgtaatgtcgcccaccctgcctcatctaccaaagtcgacaagaagatcgagcctcgaggccccactatcaaaccctgtccaccctgtaagtgccccgctccaaacttgctgggcggaccatccgttttcatcttccctccaaagatcaaagacgtgctgatgatttcactcagccctattgtcacttgtgtagtggtggacgtgtcagaagatgatcctgacgtgcagatttcctggtttgtcaacaatgttgaggtgcatacagctcagacacagacccaccgcgaagattataactctactttgagggtcgtttccgccctgccaattcagcaccaggactggatgtctggaaaggaattcaaatgtaaagtgaataataaggacctccccgctcccatcgaacggactatctctaagcctaaagggagcgtacgagctcctcaggtgtatgtcctgccccccccagaggaagaaatgaccaagaaacaggtgacccttacctgtatggttactgactttatgcctgaggacatctatgtagagtggaccaacaacgggaagactgagttgaactacaaaaacacagaacctgtgcttgatagtgatggttcttatttcatgtatagcaagctcagagtcgaaaaaaaaaactgggtggaacgcaattcttactcctgttccgtggtgcacgaggggttgcacaatcaccacactacaaaaagcttcagtaggacccccggcaag

SEQ ID NO: 60 - DNA, 639 bp, synthetic construct
  source 1..639: mol_type = other DNA
caaatcgtgctgacccagtctccagcaataatgtccgcatctcctggtgagaaagtgaccatgacttgttcagcttcctcttctgttaactatatgcactggtaccaacagaagtctggcacctccccaaagcggtggatttatgacacctccaagctggctagcggggtacccgcaaggttctccggttcaggcagcggcacttcttactccctgactattagctctatggaggcagaggatgccgctacctactattgccagcaatggagcagtaatccagtcacatttggggccggaaccaagctggagctgaagcgagctgatgcagctcccacagtatctatttttcctccatcttctgagcagctcacatctggtggggcctccgtggtctgcttcttgaataacttctatcctaaggacattaacgtgaaatggaagatcgacggatccgaacggcagaacggagtgcttaacagctggaccgaccaggatagtaaggattctacatattccatgtcttccaccctcacactcacaaaggacgagtatgagagacacaacagctacacatgtgaagccactcacaaaacctccacatctccaattgtgaagtcctttaataggaatgagtgt

SEQ ID NO: 61 - DNA, 1350 bp, synthetic construct
  source 1..1350: mol_type = other DNA
gaagttctgcttcagcagtctggcccagaagttgttaagccaggagcctccgtgaaaattacttgcaaggcctccgggtacacatttacagactacaatatggactgggtgaagcagtcccatggaaagagtctggaatggatcggcgatatcaatccaaacaatggcggtaccctctataaccagaaatttcgcggacgtgtgaccttgatcgtcgacaaaagtagttctactgcctacatggagctgcgcagcctgactagtgacgacaccgccgtctactattgcgctcgctctgaagtcttttatgggaattatgctgactactggggccagggtaccactttgaccgtctccagtgccaaaacaacagcccctagtgtatatccacttgcccctgtctgcggcgacactacagggtcttctgtgacactcgggtgtctggtcaaggggtatttccctgagccagtgaccctcacttggaactcaggctccctttctagcggcgtccacacatttccagccgtgcttcagtctgatctgtataccctgagcagcagcgtgaccgtcacctcctccacatggccttcacaaagcataacttgtaatgtcgcccaccctgcctcatctaccaaagtcgacaagaagatcgagcctcgaggccccactatcaaaccctgtccaccctgtaagtgccccgctccaaacttgctgggcggaccatccgttttcatcttccctccaaagatcaaagacgtgctgatgatttcactcagccctattgtcacttgtgtagtggtggacgtgtcagaagatgatcctgacgtgcagatttcctggtttgtcaacaatgttgaggtgcatacagctcagacacagacccaccgcgaagattataactctactttgagggtcgtttccgccctgccaattcagcaccaggactggatgtctggaaaggaattcaaatgtaaagtgaataataaggacctccccgctcccatcgaacggactatctctaagcctaaagggagcgtacgagctcctcaggtgtatgtcctgccccccccagaggaagaaatgaccaagaaacaggtgacccttacctgtatggttactgactttatgcctgaggacatctatgtagagtggaccaacaacgggaagactgagttgaactacaaaaacacagaacctgtgcttgatagtgatggttcttatttcatgtatagcaagctcagagtcgaaaaaaaaaactgggtggaacgcaattcttactcctgttccgtggtgcacgaggggttgcacaatcaccacactacaaaaagcttcagtaggacccccggcaag

SEQ ID NO: 62 - DNA, 654 bp, synthetic construct
  source 1..654: mol_type = other DNA
gacattgtgctgactcagagtcctgtaagtctggcagttcccctcggccaaagagctaccattagttgtaaggcttcccagagcgtggactatgatggcgacagctatatgaattggtatcaacagaagccaggacagccacccaagctgctgatctacgccgcctccaccctgcattcaggtatccctgtgcgattttctggtagtggctccggcacagatttcaccctgaatatccatccagttgaggaggaggatgctgcctcttactactgtcagcagagcaaagaggatcctagaaccttcggcggtggcactaagctggaaattaagcgagctgatgcagctcccacagtatctatttttcctccatcttctgagcagctcacatctggtggggcctccgtggtctgcttcttgaataacttctatcctaaggacattaacgtgaaatggaagatcgacggatccgaacggcagaacggagtgcttaacagctggaccgaccaggatagtaaggattctacatattccatgtcttccaccctcacactcacaaaggacgagtatgagagacacaacagctacacatgtgaagccactcacaaaacctccacatctccaattgtgaagtcctttaataggaatgagtgt

SEQ ID NO: 63 - DNA, 1353 bp, synthetic construct
  source 1..1353: mol_type = other DNA
gaagttcaactggttcagagcggagctgaggtaaagaagccaggtgccagcgtgaaagttagttgcaaggcatccggatacactttcactagctattatatgtattgggtgcgacaggccccagggcaaggtttggagtggatcggagagatcaatccttcaaatggcggcacaaatttcaacgaaaagttcaaatctcgcgtgactctgacagtggacaagtccatctccacagcatatatggagctgagccggcttagatccgatgacactgctgtctactattgtacaagaacactgtactatggcaacgactggtacttcgatgtctggggacaggggaccactgtgaccgtctccagtgccagtacaaagggaccatctgtgtttcctctggcaccttcatctaagagcacttctggtggtactgctgctctgggctgccttgtaaaggactatttcccagagcccgtgaccgtcagttggaattcaggcgcccttaccagcggggttcacactttcccagctgtgttgcagtcttcagggctttacagtctcagcagtgttgtcaccgtcccttcctcctcactgggcacccaaacctatatttgtaatgtcaaccataaaccaagtaacaccaaggtggacaagaaggtggagcccaagtcatgtgataaaactcacacttgtccaccatgccctgctcccgaactgttgggcggacctagcgtgtttctctttccacccaaaccaaaggataccctgatgatcagcaggactcccgaggtgacttgtgtggtggttgacgtgtcccatgaggatcctgaagtgaagttcaattggtacgtggacggcgtggaggttcataacgcaaagaccaagcccagggaagagcagtataactctacttaccgggtggtttcagtcttgactgtgttgcaccaggactggctgaatggaaaggagtataagtgtaaagtgagtaacaaagccctgccagctcccattgagaagacaatctcaaaagctaagggtcagccccgcgaaccacaggtgtatacactcccaccctcccgcgaggagatgaccaaaaaccaggtgtccctcacctgcctggtcaagggattttaccccagcgatattgctgtcgagtgggagtcaaacggtcagcccgagaataattataaaactacccctcccgtgcttgacagcgatggatctttcttcctgtactcaaaactgaccgtcgacaaatcccgatggcagcaaggtaacgtgttctcttgcagcgtaatgcacgaggctcttcacaatcactatactcagaagtcactcagccttagtcctggaaag

SEQ ID NO: 64 - DNA, 639 bp, synthetic construct
  source 1..639: mol_type = other DNA
gaaatcgtgctgacccagagcccagatttccagagtgtcacaccaaaggagaaggtaacaattacatgcagtgccagcagtagcgtgaactatatgcattggtatcagcagaaacccgatcagtcccctaagcgactgatctacgatacctccaagctggccagcggtgttccaagtaggttctctggcagcgggtctgggacagactacactctcactatcaactctctggaagctgaggatgctgctacttattattgccagcagtggagctcaaatcccgttacctttggccagggtaccaagctcgaaattaaacgtacagtcgcagcacctagtgtcttcatctttcctccctctgacgagcagttgaagagcggaactgcaagcgtcgtttgcctcctgaacaatttctatccccgggaggctaaggtccagtggaaagtggataatgctctccagagcggtaactcacaagagtctgttaccgagcaggactccaaggattctacctatagtctgagctctaccctgacactgtccaaggccgattacgagaaacacaaagtgtatgcctgcgaagtaacccaccagggcctgagttccccagtgaccaagtctttcaataggggggagtgt

SEQ ID NO: 65 - DNA, 1350 bp, synthetic construct
  source 1..1350: mol_type = other DNA
gaagtgcagcttgtacagagtggagcagaggtcaagaaaccaggagcttccgtgaaggtgagctgcaaggcctccggctatacctttactgattacaacatggactgggtccgtcaggctcctggaaaaggactggagtggattggtgacattaatcctaataacggcggcacactttacaatcagaagtttcgtggtagagttacactgactgtggataaatcaatcagcaccgcctatatggagctgtcccgactgcggtccgacgatactgcagtgtattactgcgccaggtcagaggtgttttacggtaactacgcagactattggggccaggggacaacagtgacagtcagcagcgccagtacaaagggaccatctgtgtttcctctggcaccttcatctaagagcacttctggtggtactgctgctctgggctgccttgtaaaggactatttcccagagcccgtgaccgtcagttggaattcaggcgcccttaccagcggggttcacactttcccagctgtgttgcagtcttcagggctttacagtctcagcagtgttgtcaccgtcccttcctcctcactgggcacccaaacctatatttgtaatgtcaaccataaaccaagtaacaccaaggtggacaagaaggtggagcccaagtcatgtgataaaactcacacttgtccaccatgccctgctcccgaactgttgggcggacctagcgtgtttctctttccacccaaaccaaaggataccctgatgatcagcaggactcccgaggtgacttgtgtggtggttgacgtgtcccatgaggatcctgaagtgaagttcaattggtacgtggacggcgtggaggttcataacgcaaagaccaagcccagggaagagcagtataactctacttaccgggtggtttcagtcttgactgtgttgcaccaggactggctgaatggaaaggagtataagtgtaaagtgagtaacaaagccctgccagctcccattgagaagacaatctcaaaagctaagggtcagccccgcgaaccacaggtgtatacactcccaccctcccgcgaggagatgaccaaaaaccaggtgtccctcacctgcctggtcaagggattttaccccagcgatattgctgtcgagtgggagtcaaacggtcagcccgagaataattataaaactacccctcccgtgcttgacagcgatggatctttcttcctgtactcaaaactgaccgtcgacaaatcccgatggcagcaaggtaacgtgttctcttgcagcgtaatgcacgaggctcttcacaatcactatactcagaagtcactcagccttagtcctggaaag

SEQ ID NO: 66 - DNA, 654 bp, synthetic construct
  source 1..654: mol_type = other DNA
gacatagtattgacccagacaccattgtctttgagcgttaccccaggccagccagcttcaatatcttgcaaggcctctcagtccgtcgactatgatggcgattcctacatgaattggtacctccaaaagccaggccaaccaccacagctgttgatttatgccgcttctacactccacagtggcgtgcccgatcgattttcaggatccggctcagggaccgatttcacccttaagatttctcgagtggaagccgaggatgtgggcgtgtattactgccagcagagcaaagaggatcctagaacttttggccagggaaccaagctggagattaaacgtacagtcgcagcacctagtgtcttcatctttcctccctctgacgagcagttgaagagcggaactgcaagcgtcgtttgcctcctgaacaatttctatccccgggaggctaaggtccagtggaaagtggataatgctctccagagcggtaactcacaagagtctgttaccgagcaggactccaaggattctacctatagtctgagctctaccctgacactgtccaaggccgattacgagaaacacaaagtgtatgcctgcgaagtaacccaccagggcctgagttccccagtgaccaagtctttcaataggggggagtgt